European Patent Specification EP 3 215 172 B1, published April 26, 2023. Title: MODIFICATIONS AND USES OF CONOTOXIN PEPTIDES. Applicant: Kineta Three, LLC. The sequence listing filed with the application follows.

SEQUENCE LISTING (319 sequences)

SEQ ID NO: 1 - protein, 13 aa, Conus regius
GCCSDPRCRYRCR

SEQ ID NO: 2 - protein, 13 aa, Artificial sequence
  RgIA analog
  MOD_RES (10)..(10): 3-iodo-Tyrosine
GCCSDPRCRXRCR

SEQ ID NO: 3 - protein, 13 aa, Artificial sequence
  RgIA analog
  MOD_RES (9)..(9): Citrulline
  MOD_RES (10)..(10): 3-iodo-Tyrosine
GCCTDPRCXXQCR

SEQ ID NO: 4 - protein, 15 aa, Artificial sequence
  RgIA analog
  MOD_RES (9)..(9): Citrulline
  MOD_RES (10)..(10): 3-iodo-Tyrosine
GCCTDPRCXXQCRRR

SEQ ID NO: 5 - protein, 13 aa, Artificial sequence
  RgIA analog
  MOD_RES (9)..(9): Citrulline
  MOD_RES (10)..(10): 3-iodo-Tyrosine
GCCTDPRCXXQCY

SEQ ID NO: 6 - protein, 13 aa, Artificial sequence
  RgIA analog
  MOD_RES (2)..(2): Selenocysteine
  MOD_RES (8)..(8): Selenocysteine
  MOD_RES (9)..(9): Citrulline
  MOD_RES (10)..(10): 3-iodo-Tyrosine
GXCTDPRXXXQCR

SEQ ID NO: 7 - protein, 13 aa, Artificial sequence
  RgIA analog
  MOD_RES (10)..(10): 3-iodo-Tyrosine
GCCTDPRCRXQCF

SEQ ID NO: 8 - protein, 13 aa, Artificial sequence
  RgIA analog
  MOD_RES (10)..(10): 3-iodo-Tyrosine
GCCTDPRCRXQCY

SEQ ID NO: 9 - protein, 13 aa, Artificial sequence
  RgIA analog
  MOD_RES (10)..(10): 3-iodo-Tyrosine
GCCTDPRCRXQCW

SEQ ID NO: 10 - protein, 13 aa, Artificial sequence
  RgIA analog
  VARIANT (1)..(1): des-Xaa or Gly
  VARIANT (2)..(2): des-Xaa, Cys, or selenocysteine
  VARIANT (3)..(3): des-Xaa, Cys, or selenocysteine
  VARIANT (4)..(4): des-Xaa, Ser, or Thr
  VARIANT (8)..(8): des-Xaa, Cys, or selenocysteine
  VARIANT (9)..(9): des-Xaa, Arg or citrulline
  MOD_RES (10)..(10): 3-iodo-Tyrosine
  VARIANT (11)..(11): des-Xaa, Arg, or Gln
  VARIANT (12)..(12): des-Xaa, Cys, or selenocysteine
  VARIANT (13)..(13): des-Xaa, Arg, Tyr, Phe, Trp, Tyr-Tyr, Tyr-Arg, Arg-Arg-Arg, Arg-Arg, Arg-Tyr, Arg-Arg-Tyr, or Tyr-Arg-Arg
XXXXDPRXXXXXX

SEQ ID NO: 11 - protein, 13 aa, Artificial sequence
  RgIA analog
  VARIANT (2)..(2): Cys or selenocysteine
  VARIANT (4)..(4): Ser or Thr
  VARIANT (8)..(8): Cys or selenocysteine
  VARIANT (9)..(9): Arg or citrulline
  MOD_RES (10)..(10): 3-iodo-Tyrosine
  VARIANT (11)..(11): Arg or Gln
  VARIANT (13)..(13): Arg, Tyr, Phe, Trp, or  Arg-Arg-Arg
GXCXDPRXXXXCX

SEQ ID NO: 12 - protein, 13 aa, Artificial sequence
  RgIA analog
  VARIANT (2)..(2): Cys or selenocysteine
  VARIANT (8)..(8): Cys or selenocysteine
  VARIANT (9)..(9): Arg or citrulline
  MOD_RES (10)..(10): 3-iodo-Tyrosine
  VARIANT (13)..(13): Arg or Tyr
GXCTDPRXXXQCX

SEQ ID NO: 13 - protein, 19 aa, Artificial sequence
  RgIA analog
  VARIANT (10)..(10): des-Xaa, Ser, or Thr
  MISC_FEATURE (19)..(1): Cyclization
GCCSDPRCRXRCRGAAGAG

SEQ ID NO: 14 - protein, 19 aa, Artificial sequence
  RgIA analog
  VARIANT (9)..(9): des-Xaa, Tyr, or mono-iodo-Tyr
  VARIANT (10)..(10): des-Xaa, Ser, or Thr
  MISC_FEATURE (19)..(1): Cyclization
GCCTDPRCXXQCRGAAGAG

SEQ ID NO: 15 - protein, 21 aa, Artificial sequence
  RgIA analog
  VARIANT (9)..(9): des-Xaa, Tyr, or mono-iodo-Tyr
  VARIANT (10)..(10): des-Xaa, Ser, or Thr
  MISC_FEATURE (21)..(1): Cyclization
GCCTDPRCXXQCRRRGAAGAG

SEQ ID NO: 16 - protein, 19 aa, Artificial sequence
  RgIA analog
  VARIANT (9)..(9): des-Xaa, Tyr, or mono-iodo-Tyr
  VARIANT (10)..(10): des-Xaa, Ser, or Thr
  MISC_FEATURE (19)..(1): Cyclization
GCCTDPRCXXQCYGAAGAG

SEQ ID NO: 17 - protein, 19 aa, Artificial sequence
  RgIA analog
  VARIANT (2)..(2): des-Xaa, Arg or Gln
  VARIANT (8)..(8): des-Xaa, Arg or Gln
  VARIANT (9)..(9): des-Xaa, Tyr, or mono-iodo-Tyr
  VARIANT (10)..(10): des-Xaa, Ser, or Thr
  MISC_FEATURE (19)..(1): Cyclization
GXCTDPRXXXQCRGAAGAG

SEQ ID NO: 18 - protein, 19 aa, Artificial sequence
  RgIA analog
  VARIANT (10)..(10): des-Xaa, Ser, or Thr
  MISC_FEATURE (19)..(1): Cyclization
GCCTDPRCRXQCFGAAGAG

SEQ ID NO: 19 - protein, 19 aa, Artificial sequence
  RgIA analog
  VARIANT (10)..(10): des-Xaa, Ser, or Thr
  MISC_FEATURE (19)..(1): Cyclization
GCCTDPRCRXQCYGAAGAG

SEQ ID NO: 20 - protein, 19 aa, Artificial sequence
  RgIA analog
  VARIANT (10)..(10): des-Xaa, Ser, or Thr
  MISC_FEATURE (19)..(1): Cyclization
GCCTDPRCRXQCWGAAGAG

SEQ ID NO: 21 - protein, 13 aa, Artificial sequence
  RgIA analog
  MOD_RES (13)..(13): AMIDATION
GCCSDPRCRYRCR

SEQ ID NO: 22 - protein, 13 aa, Artificial sequence
  RgIA analog
  MOD_RES (10)..(10): 3-iodo-Tyrosine
  MOD_RES (13)..(13): AMIDATION
GCCSDPRCRXRCR

SEQ ID NO: 23 - protein, 13 aa, Artificial sequence
  RgIA analog
  MOD_RES (9)..(9): Citrulline
  MOD_RES (10)..(10): 3-iodo-Tyrosine
  MOD_RES (13)..(13): AMIDATION
GCCTDPRCXXQCR

SEQ ID NO: 24 - protein, 15 aa, Artificial sequence
  RgIA analog
  MOD_RES (9)..(9): Citrulline
  MOD_RES (10)..(10): 3-iodo-Tyrosine
  MOD_RES (15)..(15): AMIDATION
GCCTDPRCXXQCRRR

SEQ ID NO: 25 - protein, 13 aa, Artificial sequence
  RgIA analog
  VARIANT (2)..(2): Cys, any natural amino acid, or any unnatural amino acid
  VARIANT (3)..(3): Cys, any natural amino acid, or any unnatural amino acid
  VARIANT (8)..(8): Cys, any natural amino acid, or any unnatural amino acid
  MOD_RES (9)..(9): Citrulline
  MOD_RES (10)..(10): 3-iodo-Tyrosine
  VARIANT (12)..(12): Cys, any natural amino acid, or any unnatural amino acid
  MOD_RES (13)..(13): AMIDATION
GXXTDPRXXXQXY

SEQ ID NO: 26 - protein, 13 aa, Artificial sequence
  RgIA analog
  MOD_RES (2)..(2): Selenocysteine
  MOD_RES (8)..(8): Selenocysteine
  MOD_RES (9)..(9): Citrulline
  MOD_RES (10)..(10): 3-iodo-Tyrosine
  MOD_RES (13)..(13): AMIDATION
GXCTDPRXXXQCR

SEQ ID NO: 27 - protein, 13 aa, Artificial sequence
  RgIA analog
  MOD_RES (10)..(10): 3-iodo-Tyrosine
  MOD_RES (13)..(13): AMIDATION
GCCTDPRCRXQCF

SEQ ID NO: 28 - protein, 13 aa, Artificial sequence
  RgIA analog
  MOD_RES (10)..(10): 3-iodo-Tyrosine
  MOD_RES (13)..(13): AMIDATION
GCCTDPRCRXQCY

SEQ ID NO: 29 - protein, 13 aa, Artificial sequence
  RgIA analog
  MOD_RES (10)..(10): 3-iodo-Tyrosine
  MOD_RES (13)..(13): AMIDATION
GCCTDPRCRXQCW

SEQ ID NO: 30 - protein, 13 aa, Artificial sequence
  RgIA analog
GCCSDPRCRYRCH

SEQ ID NO: 31 - protein, 13 aa, Artificial sequence
  RgIA analog
GCCSDPRCRYRCK

SEQ ID NO: 32 - protein, 13 aa, Artificial sequence
  RgIA analog
  VARIANT (10)..(10): O-phospho-Tyr, O-sulfo-Tyr, or O-fluoro-Tyr
GCCSDPRCRXRCR

SEQ ID NO: 33 - protein, 13 aa, Artificial sequence
  RgIA analog
  MOD_RES (1)..(1): mono-fluoro-Glycine
XCCSDPRCRYRCR

SEQ ID NO: 34 - protein, 13 aa, Artificial sequence
  RgIA analog
  MOD_RES (1)..(1): di-fluoro-Glycine
XCCSDPRCRYRCR

SEQ ID NO: 35 - protein, 13 aa, Artificial sequence
  RgIA analog
  MOD_RES (6)..(6): D-Pro
GCCSDXRCRYRCR

SEQ ID NO: 36 - protein, 13 aa, Artificial sequence
  RgIA analog
  MOD_RES (5)..(5): D-Asp
GCCSXPRCRYRCR

SEQ ID NO: 37 - protein, 13 aa, Artificial sequence
  RgIA analog
  MOD_RES (7)..(7): D-Arg
GCCSDPXCRYRCR

SEQ ID NO: 38 - protein, 13 aa, Artificial sequence
  RgIA analog
  MOD_RES (5)..(5): D-Asp
  MOD_RES (6)..(6): D-Pro
GCCSXXRCRYRCR

SEQ ID NO: 39 - protein, 13 aa, Artificial sequence
  RgIA analog
  MOD_RES (6)..(6): D-Pro
  MOD_RES (7)..(7): D-Arg
GCCSDXXCRYRCR

SEQ ID NO: 40 - protein, 13 aa, Artificial sequence
  RgIA analog
  MOD_RES (5)..(5): D-Asp
  MOD_RES (6)..(6): D-Pro
  MOD_RES (7)..(7): D-Arg
GCCSXXXCRYRCR

SEQ ID NO: 41 - protein, 13 aa, Artificial sequence
  RgIA analog
GCCSDPRCRYHCR

SEQ ID NO: 42 - protein, 13 aa, Artificial sequence
  RgIA analog
GCCSDPRCRYKCR

SEQ ID NO: 43 - protein, 13 aa, Artificial sequence
  RgIA analog
PCCSDPRCRYRCR

SEQ ID NO: 44 - protein, 13 aa, Artificial sequence
  RgIA analog
  MOD_RES (10)..(10): 3-iodo-Tyrosine
GCCSDPRCRXRCH

SEQ ID NO: 45 - protein, 13 aa, Artificial sequence
  RgIA analog
  MOD_RES (10)..(10): 3-iodo-Tyrosine
GCCSDPRCRXRCK

SEQ ID NO: 46 - protein, 13 aa, Artificial sequence
  RgIA analog
  VARIANT (10)..(10): O-phospho-Tyr, O-sulfo-Tyr, or O-fluoro-Tyr
GCCSDPRCRXRCH

SEQ ID NO: 47 - protein, 13 aa, Artificial sequence
  RgIA analog
  MOD_RES (1)..(1): mono-fluoro-Glycine
  MOD_RES (10)..(10): 3-iodo-Tyrosine
XCCSDPRCRXRCR

SEQ ID NO: 48 - protein, 13 aa, Artificial sequence
  RgIA analog
  MOD_RES (1)..(1): di-fluoro-Glycine
  MOD_RES (10)..(10): 3-iodo-Tyrosine
XCCSDPRCRXRCR

SEQ ID NO: 49 - protein, 13 aa, Artificial sequence
  RgIA analog
  MOD_RES (6)..(6): D-Pro
  MOD_RES (10)..(10): 3-iodo-Tyrosine
GCCSDXRCRXRCR

SEQ ID NO: 50 - protein, 13 aa, Artificial sequence
  RgIA analog
  MOD_RES (5)..(5): D-Asp
  MOD_RES (10)..(10): 3-iodo-Tyrosine
GCCSXPRCRXRCR

SEQ ID NO: 51 - protein, 13 aa, Artificial sequence
  RgIA analog
  MOD_RES (7)..(7): D-Arg
  MOD_RES (10)..(10): 3-iodo-Tyrosine
GCCSDPXCRXRCR

SEQ ID NO: 52 - protein, 13 aa, Artificial sequence
  RgIA analog
  MOD_RES (5)..(5): D-Asp
  MOD_RES (6)..(6): D-Pro
  MOD_RES (10)..(10): 3-iodo-Tyrosine
GCCSXXRCRXRCR

SEQ ID NO: 53 - protein, 13 aa, Artificial sequence
  RgIA analog
  MOD_RES (6)..(6): D-Pro
  MOD_RES (7)..(7): D-Arg
  MOD_RES (10)..(10): 3-iodo-Tyrosine
GCCSDXXCRXRCR

SEQ ID NO: 54 - protein, 13 aa, Artificial sequence
  RgIA analog
  MOD_RES (5)..(5): D-Asp
  MOD_RES (6)..(6): D-Pro
  MOD_RES (7)..(7): D-Arg
  MOD_RES (10)..(10): 3-iodo-Tyrosine
GCCSXXXCRXRCR

SEQ ID NO: 55 - protein, 13 aa, Artificial sequence
  RgIA analog
  MOD_RES (10)..(10): 3-iodo-Tyrosine
GCCSDPRCRXHCR

SEQ ID NO: 56 - protein, 13 aa, Artificial sequence
  RgIA analog
  MOD_RES (10)..(10): 3-iodo-Tyrosine
GCCSDPRCRXKCR

SEQ ID NO: 57 - protein, 13 aa, Artificial sequence
  RgIA analog
  MOD_RES (10)..(10): 3-iodo-Tyrosine
PCCSDPRCRXRCR

SEQ ID NO: 58 - protein, 13 aa, Artificial sequence
  RgIA analog
  MOD_RES (10)..(10): 3-iodo-Tyrosine
GCCSDPRCHXRCR

SEQ ID NO: 59 - protein, 13 aa, Artificial sequence
  RgIA analog
  MOD_RES (10)..(10): 3-iodo-Tyrosine
GCCSDPRCKXRCR

SEQ ID NO: 60 - protein, 13 aa, Artificial sequence
  RgIA analog
  MOD_RES (10)..(10): 3-iodo-Tyrosine
GCCTDPRCRXRCH

SEQ ID NO: 61 - protein, 13 aa, Artificial sequence
  RgIA analog
  MOD_RES (10)..(10): 3-iodo-Tyrosine
GCCTDPRCRXRCK

SEQ ID NO: 62 - protein, 13 aa, Artificial sequence
  RgIA analog
  VARIANT (10)..(10): O-phospho-Tyr, O-sulfo-Tyr, or O-fluoro-Tyr
GCCTDPRCRXRCR

SEQ ID NO: 63 - protein, 13 aa, Artificial sequence
  RgIA analog
  MOD_RES (1)..(1): mono-fluoro-Glycine
  MOD_RES (10)..(10): 3-iodo-Tyrosine
XCCTDPRCRXRCR

SEQ ID NO: 64 - protein, 13 aa, Artificial sequence
  RgIA analog
  MOD_RES (1)..(1): di-fluoro-Glycine
  MOD_RES (10)..(10): 3-iodo-Tyrosine
XCCTDPRCRXRCR

SEQ ID NO: 65 - protein, 13 aa, Artificial sequence
  RgIA analog
  MOD_RES (6)..(6): D-Pro
  MOD_RES (10)..(10): 3-iodo-Tyrosine
GCCTDXRCRXRCR

SEQ ID NO: 66 - protein, 13 aa, Artificial sequence
  RgIA analog
  MOD_RES (5)..(5): D-Asp
  MOD_RES (10)..(10): 3-iodo-Tyrosine
GCCTXPRCRXRCR

SEQ ID NO: 67 - protein, 13 aa, Artificial sequence
  RgIA analog
  MOD_RES (7)..(7): D-Arg
  MOD_RES (10)..(10): 3-iodo-Tyrosine
GCCTDPXCRXRCR

SEQ ID NO: 68 - protein, 13 aa, Artificial sequence
  RgIA analog
  MOD_RES (5)..(5): D-Asp
  MOD_RES (6)..(6): D-Pro
  MOD_RES (10)..(10): 3-iodo-Tyrosine
GCCTXXRCRXRCR

SEQ ID NO: 69 - protein, 13 aa, Artificial sequence
  RgIA analog
  MOD_RES (6)..(6): D-Pro
  MOD_RES (7)..(7): D-Arg
  MOD_RES (10)..(10): 3-iodo-Tyrosine
GCCTDXXCRXRCR

SEQ ID NO: 70 - protein, 13 aa, Artificial sequence
  RgIA analog
  MOD_RES (5)..(5): D-Asp
  MOD_RES (6)..(6): D-Pro
  MOD_RES (7)..(7): D-Arg
  MOD_RES (10)..(10): 3-iodo-Tyrosine
GCCTXXXCRXRCR

SEQ ID NO: 71 - protein, 13 aa, Artificial sequence
  RgIA analog
  MOD_RES (10)..(10): 3-iodo-Tyrosine
GCCTDPRCRXHCR

SEQ ID NO: 72 - protein, 13 aa, Artificial sequence
  RgIA analog
  MOD_RES (10)..(10): 3-iodo-Tyrosine
GCCTDPRCRXKCR

SEQ ID NO: 73 - protein, 13 aa, Artificial sequence
  RgIA analog
  MOD_RES (10)..(10): 3-iodo-Tyrosine
PCCTDPRCRXRCR

SEQ ID NO: 74 - protein, 13 aa, Artificial sequence
  RgIA analog
  MOD_RES (10)..(10): 3-iodo-Tyrosine
GCCTDPRCHXRCR

SEQ ID NO: 75 - protein, 13 aa, Artificial sequence
  RgIA analog
  MOD_RES (10)..(10): 3-iodo-Tyrosine
GCCTDPRCKXRCR

SEQ ID NO: 76 - protein, 15 aa, Artificial sequence
  RgIA analog
  MOD_RES (9)..(9): Citrulline
  MOD_RES (10)..(10): 3-iodo-Tyrosine
GCCTDPRCXXQCHRR

SEQ ID NO: 77 - protein, 15 aa, Artificial sequence
  RgIA analog
  MOD_RES (9)..(9): Citrulline
  MOD_RES (10)..(10): 3-iodo-Tyrosine
GCCTDPRCXXQCKRR

SEQ ID NO: 78 - protein, 15 aa, Artificial sequence
  RgIA analog
  MOD_RES (9)..(9): Citrulline
  MOD_RES (10)..(10): 3-iodo-Tyrosine
GCCTDPRCXXQCRHR

SEQ ID NO: 79 - protein, 15 aa, Artificial sequence
  RgIA analog
  MOD_RES (9)..(9): Citrulline
  MOD_RES (10)..(10): 3-iodo-Tyrosine
GCCTDPRCXXQCRKR

SEQ ID NO: 80 - protein, 15 aa, Artificial sequence
  RgIA analog
  MOD_RES (9)..(9): Citrulline
  MOD_RES (10)..(10): 3-iodo-Tyrosine
GCCTDPRCXXQCRRH

SEQ ID NO: 81 - protein, 15 aa, Artificial sequence
  RgIA analog
  MOD_RES (9)..(9): Citrulline
  MOD_RES (10)..(10): 3-iodo-Tyrosine
GCCTDPRCXXQCRRK

SEQ ID NO: 82 - protein, 15 aa, Artificial sequence
  RgIA analog
  MOD_RES (9)..(9): Citrulline
  VARIANT (10)..(10): O-phospho-Tyr, O-sulfo-Tyr, or O-fluoro-Tyr
GCCTDPRCXXQCRRR

SEQ ID NO: 83 - protein, 15 aa, Artificial sequence
  RgIA analog
  MOD_RES (1)..(1): mono-fluoro-Glycine
  MOD_RES (9)..(9): Citrulline
  MOD_RES (10)..(10): 3-iodo-Tyrosine
XCCTDPRCXXQCRRR

SEQ ID NO: 84 - protein, 15 aa, Artificial sequence
  RgIA analog
  MOD_RES (1)..(1): di-fluoro-Glycine
  MOD_RES (9)..(9): Citrulline
  MOD_RES (10)..(10): 3-iodo-Tyrosine
XCCTDPRCXXQCRRR

SEQ ID NO: 85 - protein, 15 aa, Artificial sequence
  RgIA analog
  MOD_RES (6)..(6): D-Pro
  MOD_RES (9)..(9): Citrulline
  MOD_RES (10)..(10): 3-iodo-Tyrosine
GCCTDXRCXXQCRRR

SEQ ID NO: 86 - protein, 15 aa, Artificial sequence
  RgIA analog
  MOD_RES (5)..(5): D-Asp
  MOD_RES (9)..(9): Citrulline
  MOD_RES (10)..(10): 3-iodo-Tyrosine
GCCTXPRCXXQCRRR

SEQ ID NO: 87 - protein, 15 aa, Artificial sequence
  RgIA analog
  MOD_RES (7)..(7): D-Arg
  MOD_RES (9)..(9): Citrulline
  MOD_RES (10)..(10): 3-iodo-Tyrosine
GCCTDPXCXXQCRRR

SEQ ID NO: 88 - protein, 15 aa, Artificial sequence
  RgIA analog
  MOD_RES (5)..(5): D-Asp
  MOD_RES (6)..(6): D-Pro
  MOD_RES (9)..(9): Citrulline
  MOD_RES (10)..(10): 3-iodo-Tyrosine
GCCTXXRCXXQCRRR

SEQ ID NO: 89 - protein, 15 aa, Artificial sequence
  RgIA analog
  MOD_RES (6)..(6): D-Pro
  MOD_RES (7)..(7): D-Arg
  MOD_RES (9)..(9): Citrulline
  MOD_RES (10)..(10): 3-iodo-Tyrosine
GCCTDXXCXXQCRRR

SEQ ID NO: 90 - protein, 15 aa, Artificial sequence
  RgIA analog
  MOD_RES (5)..(5): D-Asp
  MOD_RES (6)..(6): D-Pro
  MOD_RES (7)..(7): D-Arg
  MOD_RES (9)..(9): Citrulline
  MOD_RES (10)..(10): 3-iodo-Tyrosine
GCCTXXXCXXQCRRR

SEQ ID NO: 91 - protein, 15 aa, Artificial sequence
  RgIA analog
  MOD_RES (9)..(9): Citrulline
  MOD_RES (10)..(10): 3-iodo-Tyrosine
PCCTDPRCXXQCRRR

SEQ ID NO: 92 - protein, 13 aa, Artificial sequence
  RgIA analog
  MOD_RES (9)..(9): Citrulline
  VARIANT (10)..(10): O-phospho-Tyr, O-sulfo-Tyr, or O-fluoro-Tyr
GCCTDPRCXXQCY

SEQ ID NO: 93 - protein, 13 aa, Artificial sequence
  RgIA analog
  MOD_RES (9)..(9): Citrulline
  MOD_RES (10)..(10): 3-iodo-Tyrosine
  VARIANT (13)..(13): O-phospho-Tyr, O-sulfo-Tyr, or O-fluoro-Tyr
GCCTDPRCXXQCX

SEQ ID NO: 94 - protein, 13 aa, Artificial sequence
  RgIA analog
  MOD_RES (1)..(1): mono-fluoro-Glycine
  MOD_RES (9)..(9): Citrulline
  MOD_RES (10)..(10): 3-iodo-Tyrosine
XCCTDPRCXXQCY

SEQ ID NO: 95 - protein, 13 aa, Artificial sequence
  RgIA analog
  MOD_RES (1)..(1): di-fluoro-Glycine
  MOD_RES (9)..(9): Citrulline
  MOD_RES (10)..(10): 3-iodo-Tyrosine
XCCTDPRCXXQCY

SEQ ID NO: 96 - protein, 13 aa, Artificial sequence
  RgIA analog
  MOD_RES (6)..(6): D-Pro
  MOD_RES (9)..(9): Citrulline
  MOD_RES (10)..(10): 3-iodo-Tyrosine
GCCTDXRCXXQCY

SEQ ID NO: 97 - protein, 13 aa, Artificial sequence
  RgIA analog
  MOD_RES (5)..(5): D-Asp
  MOD_RES (9)..(9): Citrulline
  MOD_RES (10)..(10): 3-iodo-Tyrosine
GCCTXPRCXXQCY

SEQ ID NO: 98 - protein, 13 aa, Artificial sequence
  RgIA analog
  MOD_RES (7)..(7): D-Arg
  MOD_RES (9)..(9): Citrulline
  MOD_RES (10)..(10): 3-iodo-Tyrosine
GCCTDPXCXXQCY

SEQ ID NO: 99 - protein, 13 aa, Artificial sequence
  RgIA analog
  MOD_RES (5)..(5): D-Asp
  MOD_RES (6)..(6): D-Pro
  MOD_RES (9)..(9): Citrulline
  MOD_RES (10)..(10): 3-iodo-Tyrosine
GCCTXXRCXXQCY

SEQ ID NO: 100 - protein, 13 aa, Artificial sequence
  RgIA analog
  MOD_RES (6)..(6): D-Pro
  MOD_RES (7)..(7): D-Arg
  MOD_RES (9)..(9): Citrulline
  MOD_RES (10)..(10): 3-iodo-Tyrosine
GCCTDXXCXXQCY

SEQ ID NO: 101 - protein, 13 aa, Artificial sequence
  RgIA analog
  MOD_RES (5)..(5): D-Asp
  MOD_RES (6)..(6): D-Pro
  MOD_RES (7)..(7): D-Arg
  MOD_RES (9)..(9): Citrulline
  MOD_RES (10)..(10): 3-iodo-Tyrosine
GCCTXXXCXXQCY

SEQ ID NO: 102 - protein, 13 aa, Artificial sequence
  RgIA analog
  MOD_RES (9)..(9): Citrulline
  MOD_RES (10)..(10): 3-iodo-Tyrosine
PCCTDPRCXXQCY

SEQ ID NO: 103 - protein, 13 aa, Artificial sequence
  RgIA analog
  MOD_RES (2)..(2): Selenocysteine
  MOD_RES (8)..(8): Selenocysteine
  MOD_RES (9)..(9): Citrulline
  MOD_RES (10)..(10): 3-iodo-Tyrosine
GXCTDPRXXXQCH

SEQ ID NO: 104 - protein, 13 aa, Artificial sequence
  RgIA analog
  MOD_RES (2)..(2): Selenocysteine
  MOD_RES (8)..(8): Selenocysteine
  MOD_RES (9)..(9): Citrulline
  MOD_RES (10)..(10): 3-iodo-Tyrosine
GXCTDPRXXXQCK

SEQ ID NO: 105 - protein, 13 aa, Artificial sequence
  RgIA analog
  MOD_RES (2)..(2): Selenocysteine
  MOD_RES (8)..(8): Selenocysteine
  MOD_RES (9)..(9): Citrulline
  VARIANT (10)..(10): O-phospho-Tyr, O-sulfo-Tyr, or O-fluoro-Tyr
GXCTDPRXXXQCR

SEQ ID NO: 106 - protein, 13 aa, Artificial sequence
  RgIA analog
  MOD_RES (1)..(1): mono-fluoro-Glycine
  MOD_RES (2)..(2): Selenocysteine
  MOD_RES (8)..(8): Selenocysteine
  MOD_RES (9)..(9): Citrulline
  MOD_RES (10)..(10): 3-iodo-Tyrosine
XXCTDPRXXXQCR

SEQ ID NO: 107 - protein, 13 aa, Artificial sequence
  RgIA analog
  MOD_RES (1)..(1): di-fluoro-Glycine
  MOD_RES (2)..(2): Selenocysteine
  MOD_RES (8)..(8): Selenocysteine
  MOD_RES (9)..(9): Citrulline
  MOD_RES (10)..(10): 3-iodo-Tyrosine
XXCTDPRXXXQCR

SEQ ID NO: 108 - protein, 13 aa, Artificial sequence
  RgIA analog
  MOD_RES (2)..(2): Selenocysteine
  MOD_RES (6)..(6): D-Pro
  MOD_RES (8)..(8): Selenocysteine
  MOD_RES (9)..(9): Citrulline
  MOD_RES (10)..(10): 3-iodo-Tyrosine
GXCTDXRXXXQCR

SEQ ID NO: 109 - protein, 13 aa, Artificial sequence
  RgIA analog
  MOD_RES (2)..(2): Selenocysteine
  MOD_RES (5)..(5): D-Asp
  MOD_RES (8)..(8): Selenocysteine
  MOD_RES (9)..(9): Citrulline
  MOD_RES (10)..(10): 3-iodo-Tyrosine
GXCTXPRXXXQCR

SEQ ID NO: 110 - protein, 13 aa, Artificial sequence
  RgIA analog
  MOD_RES (2)..(2): Selenocysteine
  MOD_RES (7)..(7): D-Arg
  MOD_RES (8)..(8): Selenocysteine
  MOD_RES (9)..(9): Citrulline
  MOD_RES (10)..(10): 3-iodo-Tyrosine
GXCTDPXXXXQCR

SEQ ID NO: 111 - protein, 13 aa, Artificial sequence
  RgIA analog
  MOD_RES (2)..(2): Selenocysteine
  MOD_RES (5)..(5): D-Asp
  MOD_RES (6)..(6): D-Pro
  MOD_RES (8)..(8): Selenocysteine
  MOD_RES (9)..(9): Citrulline
  MOD_RES (10)..(10): 3-iodo-Tyrosine
GXCTXXRXXXQCR

SEQ ID NO: 112 - protein, 13 aa, Artificial sequence
  RgIA analog
  MOD_RES (2)..(2): Selenocysteine
  MOD_RES (6)..(6): D-Pro
  MOD_RES (7)..(7): D-Arg
  MOD_RES (8)..(8): Selenocysteine
  MOD_RES (9)..(9): Citrulline
  MOD_RES (10)..(10): 3-iodo-Tyrosine
GXCTDXXXXXQCR

SEQ ID NO: 113 - protein, 13 aa, Artificial sequence
  RgIA analog
  MOD_RES (2)..(2): Selenocysteine
  MOD_RES (5)..(5): D-Asp
  MOD_RES (6)..(6): D-Pro
  MOD_RES (7)..(7): D-Arg
  MOD_RES (8)..(8): Selenocysteine
  MOD_RES (9)..(9): Citrulline
  MOD_RES (10)..(10): 3-iodo-Tyrosine
GXCTXXXXXXQCR

SEQ ID NO: 114 - protein, 13 aa, Artificial sequence
  RgIA analog
  MOD_RES (2)..(2): Selenocysteine
  MOD_RES (8)..(8): Selenocysteine
  MOD_RES (9)..(9): Citrulline
  MOD_RES (10)..(10): 3-iodo-Tyrosine
PXCTDPRXXXQCR

SEQ ID NO: 115 - protein, 13 aa, Artificial sequence
  RgIA analog
  VARIANT (10)..(10): O-phospho-Tyr, O-sulfo-Tyr, or O-fluoro-Tyr
GCCTDPRCRXQCF

SEQ ID NO: 116 - protein, 13 aa, Artificial sequence
  RgIA analog
  MOD_RES (1)..(1): mono-fluoro-Glycine
  MOD_RES (10)..(10): 3-iodo-Tyrosine
XCCTDPRCRXQCF

SEQ ID NO: 117 - protein, 13 aa, Artificial sequence
  RgIA analog
  MOD_RES (1)..(1): di-fluoro-Glycine
  MOD_RES (10)..(10): 3-iodo-Tyrosine
XCCTDPRCRXQCF

SEQ ID NO: 118 - protein, 13 aa, Artificial sequence
  RgIA analog
  MOD_RES (6)..(6): D-Pro
  MOD_RES (10)..(10): 3-iodo-Tyrosine
GCCTDXRCRXQCF

SEQ ID NO: 119 - protein, 13 aa, Artificial sequence
  RgIA analog
  MOD_RES (5)..(5): D-Asp
  MOD_RES (10)..(10): 3-iodo-Tyrosine
GCCTXPRCRXQCF

SEQ ID NO: 120 - protein, 13 aa, Artificial sequence
  RgIA analog
  MOD_RES (7)..(7): D-Arg
  MOD_RES (10)..(10): 3-iodo-Tyrosine
GCCTDPXCRXQCF

SEQ ID NO: 121 - protein, 13 aa, Artificial sequence
  RgIA analog
  MOD_RES (5)..(5): D-Asp
  MOD_RES (6)..(6): D-Pro
  MOD_RES (10)..(10): 3-iodo-Tyrosine
GCCTXXRCRXQCF

SEQ ID NO: 122 - protein, 13 aa, Artificial sequence
  RgIA analog
  MOD_RES (6)..(6): D-Pro
  MOD_RES (7)..(7): D-Arg
  MOD_RES (10)..(10): 3-iodo-Tyrosine
GCCTDXXCRXQCF

SEQ ID NO: 123 - protein, 13 aa, Artificial sequence
  RgIA analog
  MOD_RES (5)..(5): D-Asp
  MOD_RES (6)..(6): D-Pro
  MOD_RES (7)..(7): D-Arg
  MOD_RES (10)..(10): 3-iodo-Tyrosine
GCCTXXXCRXQCF

SEQ ID NO: 124 - protein, 13 aa, Artificial sequence
  RgIA analog
  MOD_RES (10)..(10): 3-iodo-Tyrosine
PCCTDPRCRXQCF

SEQ ID NO: 125 - protein, 13 aa, Artificial sequence
  RgIA analog
  VARIANT (10)..(10): O-phospho-Tyr, O-sulfo-Tyr, or O-fluoro-Tyr
GCCTDPRCRXQCY

SEQ ID NO: 126 - protein, 13 aa, Artificial sequence
  RgIA analog
  MOD_RES (10)..(10): 3-iodo-Tyrosine
  VARIANT (13)..(13): O-phospho-Tyr, O-sulfo-Tyr, or O-fluoro-Tyr
GCCTDPRCRXQCX

SEQ ID NO: 127 - protein, 13 aa, Artificial sequence
  RgIA analog
  MOD_RES (1)..(1): mono-fluoro-Glycine
  MOD_RES (10)..(10): 3-iodo-Tyrosine
XCCTDPRCRXQCY

SEQ ID NO: 128 - protein, 13 aa, Artificial sequence
  RgIA analog
  MOD_RES (1)..(1): di-fluoro-Glycine
  MOD_RES (10)..(10): 3-iodo-Tyrosine
XCCTDPRCRXQCY

SEQ ID NO: 129 - protein, 13 aa, Artificial sequence
  RgIA analog
  MOD_RES (6)..(6): D-Pro
  MOD_RES (10)..(10): 3-iodo-Tyrosine
GCCTDXRCRXQCY

SEQ ID NO: 130 - protein, 13 aa, Artificial sequence
  RgIA analog
  MOD_RES (5)..(5): D-Asp
  MOD_RES (10)..(10): 3-iodo-Tyrosine
GCCTXPRCRXQCY

SEQ ID NO: 131 - protein, 13 aa, Artificial sequence
  RgIA analog
  MOD_RES (7)..(7): D-Arg
  MOD_RES (10)..(10): 3-iodo-Tyrosine
GCCTDPXCRXQCY

SEQ ID NO: 132 - protein, 13 aa, Artificial sequence
  RgIA analog
  MOD_RES (5)..(5): D-Asp
  MOD_RES (6)..(6): D-Pro
  MOD_RES (10)..(10): 3-iodo-Tyrosine
GCCTXXRCRXQCY

SEQ ID NO: 133 - protein, 13 aa, Artificial sequence
  RgIA analog
  MOD_RES (6)..(6): D-Pro
  MOD_RES (7)..(7): D-Arg
  MOD_RES (10)..(10): 3-iodo-Tyrosine
GCCTDXXCRXQCY

SEQ ID NO: 134 - protein, 13 aa, Artificial sequence
  RgIA analog
  MOD_RES (5)..(5): D-Asp
  MOD_RES (6)..(6): D-Pro
  MOD_RES (7)..(7): D-Arg
  MOD_RES (10)..(10): 3-iodo-Tyrosine
GCCTXXXCRXQCY

SEQ ID NO: 135 - protein, 13 aa, Artificial sequence
  RgIA analog
  MOD_RES (10)..(10): 3-iodo-Tyrosine
PCCTDPRCRXQCY

SEQ ID NO: 136 - protein, 13 aa, Artificial sequence
  RgIA analog
  VARIANT (10)..(10): O-phospho-Tyr, O-sulfo-Tyr, or O-fluoro-Tyr
GCCTDPRCRXQCW

SEQ ID NO: 137 - protein, 13 aa, Artificial sequence
  RgIA analog
  MOD_RES (1)..(1): mono-fluoro-Glycine
  MOD_RES (10)..(10): 3-iodo-Tyrosine
XCCTDPRCRXQCW

SEQ ID NO: 138 - protein, 13 aa, Artificial sequence
  RgIA analog
  MOD_RES (1)..(1): di-fluoro-Glycine
  MOD_RES (10)..(10): 3-iodo-Tyrosine
XCCTDPRCRXQCW

SEQ ID NO: 139 - protein, 13 aa, Artificial sequence
  RgIA analog
  MOD_RES (6)..(6): D-Pro
  MOD_RES (10)..(10): 3-iodo-Tyrosine
GCCTDXRCRXQCW

SEQ ID NO: 140 - protein, 13 aa, Artificial sequence
  RgIA analog
  MOD_RES (5)..(5): D-Asp
  MOD_RES (10)..(10): 3-iodo-Tyrosine
GCCTXPRCRXQCW

SEQ ID NO: 141 - protein, 13 aa, Artificial sequence
  RgIA analog
  MOD_RES (7)..(7): D-Arg
  MOD_RES (10)..(10): 3-iodo-Tyrosine
GCCTDPXCRXQCW

SEQ ID NO: 142 - protein, 13 aa, Artificial sequence
  RgIA analog
  MOD_RES (5)..(5): D-Asp
  MOD_RES (6)..(6): D-Pro
  MOD_RES (10)..(10): 3-iodo-Tyrosine
GCCTXXRCRXQCW

SEQ ID NO: 143 - protein, 13 aa, Artificial sequence
  RgIA analog
  MOD_RES (6)..(6): D-Pro
  MOD_RES (7)..(7): D-Arg
  MOD_RES (10)..(10): 3-iodo-Tyrosine
GCCTDXXCRXQCW

SEQ ID NO: 144 - protein, 13 aa, Artificial sequence
  RgIA analog
  MOD_RES (5)..(5): D-Asp
  MOD_RES (6)..(6): D-Pro
  MOD_RES (7)..(7): D-Arg
  MOD_RES (10)..(10): 3-iodo-Tyrosine
GCCTXXXCRXQCW

SEQ ID NO: 145 - protein, 13 aa, Artificial sequence
  RgIA analog
  MOD_RES (10)..(10): 3-iodo-Tyrosine
PCCTDPRCRXQCW

SEQ ID NO: 146 - protein, 13 aa, Artificial sequence
  RgIA analog
  MOD_RES (2)..(2): Selenocysteine
  MOD_RES (9)..(9): Citrulline
  MOD_RES (10)..(10): 3-iodo-Tyrosine
GXCTDPRCXXQCY

SEQ ID NO: 147 - protein, 13 aa, Artificial sequence
  RgIA analog
  MOD_RES (3)..(3): Selenocysteine
  MOD_RES (9)..(9): Citrulline
  MOD_RES (10)..(10): 3-iodo-Tyrosine
GCXTDPRCXXQCY

SEQ ID NO: 148 - protein, 13 aa, Artificial sequence
  RgIA analog
  MOD_RES (8)..(8): Selenocysteine
  MOD_RES (9)..(9): Citrulline
  MOD_RES (10)..(10): 3-iodo-Tyrosine
GCCTDPRXXXQCY

SEQ ID NO: 149 - protein, 13 aa, Artificial sequence
  RgIA analog
  MOD_RES (9)..(9): Citrulline
  MOD_RES (10)..(10): 3-iodo-Tyrosine
  MOD_RES (12)..(12): Selenocysteine
GCCTDPRCXXQXY

SEQ ID NO: 150 - protein, 13 aa, Artificial sequence
  RgIA analog
  MOD_RES (2)..(2): Selenocysteine
  MOD_RES (8)..(8): Selenocysteine
  MOD_RES (9)..(9): Citrulline
  MOD_RES (10)..(10): 3-iodo-Tyrosine
GXCTDPRXXXQCY

SEQ ID NO: 151 - protein, 13 aa, Artificial sequence
  RgIA analog
  MOD_RES (3)..(3): Selenocysteine
  MOD_RES (9)..(9): Citrulline
  MOD_RES (10)..(10): 3-iodo-Tyrosine
  MOD_RES (12)..(12): Selenocysteine
GCXTDPRCXXQXY

SEQ ID NO: 152 - protein, 13 aa, Artificial sequence
  RgIA analog
  MOD_RES (2)..(2): Selenocysteine
  MOD_RES (3)..(3): Selenocysteine
  MOD_RES (9)..(9): Citrulline
  MOD_RES (10)..(10): 3-iodo-Tyrosine
GXXTDPRCXXQCY

SEQ ID NO: 153 - protein, 13 aa, Artificial sequence
  RgIA analog
  MOD_RES (8)..(8): Selenocysteine
  MOD_RES (9)..(9): Citrulline
  MOD_RES (10)..(10): 3-iodo-Tyrosine
  MOD_RES (12)..(12): Selenocysteine
GCCTDPRXXXQXY

SEQ ID NO: 154 - protein, 13 aa, Artificial sequence
  RgIA analog
  MOD_RES (2)..(2): Selenocysteine
  MOD_RES (9)..(9): Citrulline
  MOD_RES (10)..(10): 3-iodo-Tyrosine
  MOD_RES (12)..(12): Selenocysteine
GXCTDPRCXXQXY

SEQ ID NO: 155 - protein, 13 aa, Artificial sequence
  RgIA analog
  MOD_RES (2)..(2): Selenocysteine
  MOD_RES (3)..(3): Selenocysteine
  MOD_RES (8)..(8): Selenocysteine
  MOD_RES (9)..(9): Citrulline
  MOD_RES (10)..(10): 3-iodo-Tyrosine
GXXTDPRXXXQCY

SEQ ID NO: 156 - protein, 13 aa, Artificial sequence
  RgIA analog
  MOD_RES (3)..(3): Selenocysteine
  MOD_RES (8)..(8): Selenocysteine
  MOD_RES (9)..(9): Citrulline
  MOD_RES (10)..(10): 3-iodo-Tyrosine
  MOD_RES (12)..(12): Selenocysteine
GCXTDPRXXXQXY

SEQ ID NO: 157 - protein, 13 aa, Artificial sequence
  RgIA analog
  MOD_RES (2)..(2): Selenocysteine
  MOD_RES (8)..(8): Selenocysteine
  MOD_RES (9)..(9): Citrulline
  MOD_RES (10)..(10): 3-iodo-Tyrosine
  MOD_RES (12)..(12): Selenocysteine
GXCTDPRXXXQXY

SEQ ID NO: 158 - protein, 13 aa, Artificial sequence
  RgIA analog
  MOD_RES (2)..(2): Selenocysteine
  MOD_RES (3)..(3): Selenocysteine
  MOD_RES (9)..(9): Citrulline
  MOD_RES (10)..(10): 3-iodo-Tyrosine
  MOD_RES (12)..(12): Selenocysteine
GXXTDPRCXXQXY

SEQ ID NO: 159 - protein, 13 aa, Artificial sequence
  RgIA analog
  MOD_RES (2)..(2): Selenocysteine
  MOD_RES (3)..(3): Selenocysteine
  MOD_RES (8)..(8): Selenocysteine
  MOD_RES (9)..(9): Citrulline
  MOD_RES (10)..(10): 3-iodo-Tyrosine
  MOD_RES (12)..(12): Selenocysteine
GXXTDPRXXXQXY

SEQ ID NO: 160 - protein, 13 aa, Artificial sequence
  RgIA analog
  MOD_RES (2)..(2): Selenocysteine
  MOD_RES (10)..(10): 3-iodo-Tyrosine
GXCTDPRCRXQCY

SEQ ID NO: 161 - protein, 13 aa, Artificial sequence
  RgIA analog
  MOD_RES (3)..(3): Selenocysteine
  MOD_RES (10)..(10): 3-iodo-Tyrosine
GCXTDPRCRXQCY

SEQ ID NO: 162 - protein, 13 aa, Artificial sequence
  RgIA analog
  MOD_RES (8)..(8): Selenocysteine
  MOD_RES (10)..(10): 3-iodo-Tyrosine
GCCTDPRXRXQCY

SEQ ID NO: 163 - protein, 13 aa, Artificial sequence
  RgIA analog
  MOD_RES (10)..(10): 3-iodo-Tyrosine
  MOD_RES (12)..(12): Selenocysteine
GCCTDPRCRXQXY

SEQ ID NO: 164 - protein, 13 aa, Artificial sequence
  RgIA analog
  MOD_RES (2)..(2): Selenocysteine
  MOD_RES (8)..(8): Selenocysteine
  MOD_RES (10)..(10): 3-iodo-Tyrosine
GXCTDPRXRXQCY

SEQ ID NO: 165 - protein, 13 aa, Artificial sequence
  RgIA analog
  MOD_RES (3)..(3): Selenocysteine
  MOD_RES (10)..(10): 3-iodo-Tyrosine
  MOD_RES (12)..(12): Selenocysteine
GCXTDPRCRXQXY

SEQ ID NO: 166 - protein, 13 aa, Artificial sequence
  RgIA analog
  MOD_RES (2)..(2): Selenocysteine
  MOD_RES (3)..(3): Selenocysteine
  MOD_RES (10)..(10): 3-iodo-Tyrosine
GXXTDPRCRXQCY

SEQ ID NO: 167 - protein, 13 aa, Artificial sequence
  RgIA analog
  MOD_RES (8)..(8): Selenocysteine
  MOD_RES (10)..(10): 3-iodo-Tyrosine
  MOD_RES (12)..(12): Selenocysteine
GCCTDPRXRXQXY

SEQ ID NO: 168 - protein, 13 aa, Artificial sequence
  RgIA analog
  MOD_RES (2)..(2): Selenocysteine
  MOD_RES (10)..(10): 3-iodo-Tyrosine
  MOD_RES (12)..(12): Selenocysteine
GXCTDPRCRXQXY

SEQ ID NO: 169 - protein, 13 aa, Artificial sequence
  RgIA analog
  MOD_RES (2)..(2): Selenocysteine
  MOD_RES (3)..(3): Selenocysteine
  MOD_RES (8)..(8): Selenocysteine
  MOD_RES (10)..(10): 3-iodo-Tyrosine
GXXTDPRXRXQCY

SEQ ID NO: 170 - protein, 13 aa, Artificial sequence
  RgIA analog
  MOD_RES (3)..(3): Selenocysteine
  MOD_RES (8)..(8): Selenocysteine
  MOD_RES (10)..(10): 3-iodo-Tyrosine
  MOD_RES (12)..(12): Selenocysteine
GCXTDPRXRXQXY

SEQ ID NO: 171 - protein, 13 aa, Artificial sequence
  RgIA analog
  MOD_RES (2)..(2): Selenocysteine
  MOD_RES (8)..(8): Selenocysteine
  MOD_RES (10)..(10): 3-iodo-Tyrosine
  MOD_RES (12)..(12): Selenocysteine
GXCTDPRXRXQXY

SEQ ID NO: 172 - protein, 13 aa, Artificial sequence
  RgIA analog
  MOD_RES (2)..(2): Selenocysteine
  MOD_RES (3)..(3): Selenocysteine
  MOD_RES (10)..(10): 3-iodo-Tyrosine
  MOD_RES (12)..(12): Selenocysteine
GXXTDPRCRXQXY

SEQ ID NO: 173 - protein, 13 aa, Artificial sequence
  RgIA analog
  MOD_RES (2)..(2): Selenocysteine
  MOD_RES (3)..(3): Selenocysteine
  MOD_RES (8)..(8): Selenocysteine
  MOD_RES (10)..(10): 3-iodo-Tyrosine
  MOD_RES (12)..(12): Selenocysteine
GXXTDPRXRXQXY

SEQ ID NO: 174 - protein, 14 aa, Artificial sequence
  RgIA analog
  VARIANT (1)..(1): des-Xaa or Gly
  VARIANT (2)..(2): des-Xaa, Cys, or selenocysteine
  VARIANT (3)..(3): des-Xaa, Cys, or selenocysteine
  VARIANT (4)..(4): des-Xaa, Ser, or Thr
  MISC_FEATURE (5)..(5): 2-amino ethoxyacetic acid
  VARIANT (9)..(9): des-Xaa, Cys, or selenocysteine
  VARIANT (10)..(10): des-Xaa, Arg, citrulline, or omega-nitro-Arg
  VARIANT (11)..(11): des-Xaa, Tyr, or mono-iodo-Tyr
  VARIANT (12)..(12): des-Xaa, Arg, or Gln
  VARIANT (13)..(13): des-Xaa, Cys, or selenocysteine
  VARIANT (14)..(14): des-Xaa, Arg, Tyr, Phe, Trp, Tyr-Tyr, Tyr-Arg, Arg-Arg-Arg, Arg-Arg, Arg-Tyr, Arg-Arg-Tyr, or Tyr-Arg-Arg
XXXXXDPRXXXXXX

SEQ ID NO: 175 - protein, 14 aa, Artificial sequence
  RgIA analog
  VARIANT (1)..(1): des-Xaa or Gly
  VARIANT (2)..(2): des-Xaa, Cys, or selenocysteine
  VARIANT (3)..(3): des-Xaa, Cys, or selenocysteine
  VARIANT (4)..(4): des-Xaa, Ser, or Thr
  MISC_FEATURE (6)..(6): 2-amino ethoxyacetic acid
  VARIANT (9)..(9): des-Xaa, Cys, or selenocysteine
  VARIANT (10)..(10): des-Xaa, Arg, citrulline, or omega-nitro-Arg
  VARIANT (11)..(11): des-Xaa, Tyr, or mono-iodo-Tyr
  VARIANT (12)..(12): des-Xaa, Arg, or Gln
  VARIANT (13)..(13): des-Xaa, Cys, or selenocysteine
  VARIANT (14)..(14): des-Xaa, Arg, Tyr, Phe, Trp, Tyr-Tyr, Tyr-Arg, Arg-Arg-Arg, Arg-Arg, Arg-Tyr, Arg-Arg-Tyr, or Tyr-Arg-Arg
XXXXDXPRXXXXXX

SEQ ID NO: 176 - protein, 14 aa, Artificial sequence
  RgIA analog
  VARIANT (1)..(1): des-Xaa or Gly
  VARIANT (2)..(2): des-Xaa, Cys, or selenocysteine
  VARIANT (3)..(3): des-Xaa, Cys, or selenocysteine
  VARIANT (4)..(4): des-Xaa, Ser, or Thr
  MISC_FEATURE (7)..(7): 2-amino ethoxyacetic acid
  VARIANT (9)..(9): des-Xaa, Cys, or selenocysteine
  VARIANT (10)..(10): des-Xaa, Arg, citrulline, or omega-nitro-Arg
  VARIANT (11)..(11): des-Xaa, Tyr, or mono-iodo-Tyr
  VARIANT (12)..(12): des-Xaa, Arg, or Gln
  VARIANT (13)..(13): des-Xaa, Cys, or selenocysteine
  VARIANT (14)..(14): des-Xaa, Arg, Tyr, Phe, Trp, Tyr-Tyr, Tyr-Arg, Arg-Arg-Arg, Arg-Arg, Arg-Tyr, Arg-Arg-Tyr, or Tyr-Arg-Arg
XXXXDPXRXXXXXX

SEQ ID NO: 177 - protein, 14 aa, Artificial sequence
  RgIA analog
  VARIANT (1)..(1): des-Xaa or Gly
  VARIANT (2)..(2): des-Xaa, Cys, or selenocysteine
  VARIANT (3)..(3): des-Xaa, Cys, or selenocysteine
  VARIANT (4)..(4): des-Xaa, Ser, or Thr
  MISC_FEATURE (8)..(8): 2-amino ethoxyacetic acid
  VARIANT (9)..(9): des-Xaa, Cys, or selenocysteine
  VARIANT (10)..(10): des-Xaa, Arg, citrulline, or omega-nitro-Arg
  VARIANT (11)..(11): des-Xaa, Tyr, or mono-iodo-Tyr
  VARIANT (12)..(12): des-Xaa, Arg, or Gln
  VARIANT (13)..(13): des-Xaa, Cys, or selenocysteine
  VARIANT (14)..(14): des-Xaa, Arg, Tyr, Phe, Trp, Tyr-Tyr, Tyr-Arg, Arg-Arg-Arg, Arg-Arg, Arg-Tyr, Arg-Arg-Tyr, or Tyr-Arg-Arg
XXXXDPRXXXXXXX

SEQ ID NO: 178 - protein, 14 aa, Artificial sequence
  RgIA analog
  VARIANT (1)..(1): des-Xaa or Gly
  VARIANT (2)..(2): des-Xaa, Cys, or selenocysteine
  VARIANT (3)..(3): des-Xaa, Cys, or selenocysteine
  VARIANT (4)..(4): des-Xaa, Ser, or Thr
  MISC_FEATURE (5)..(5): 2-[2-[ethoxy]ethoxy]acetic acid
  VARIANT (9)..(9): des-Xaa, Cys, or selenocysteine
  VARIANT (10)..(10): des-Xaa, Arg, citrulline, or omega-nitro-Arg
  VARIANT (11)..(11): des-Xaa, Tyr, or mono-iodo-Tyr
  VARIANT (12)..(12): des-Xaa, Arg, or Gln
  VARIANT (13)..(13): des-Xaa, Cys, or selenocysteine
  VARIANT (14)..(14): des-Xaa, Arg, Tyr, Phe, Trp, Tyr-Tyr, Tyr-Arg, Arg-Arg-Arg, Arg-Arg, Arg-Tyr, Arg-Arg-Tyr, or Tyr-Arg-Arg
XXXXXDPRXXXXXX

SEQ ID NO: 179 - protein, 14 aa, Artificial sequence
  RgIA analog
  VARIANT (1)..(1): des-Xaa or Gly
  VARIANT (2)..(2): des-Xaa, Cys, or selenocysteine
  VARIANT (3)..(3): des-Xaa, Cys, or selenocysteine
  VARIANT (4)..(4): des-Xaa, Ser, or Thr
  MISC_FEATURE (6)..(6): 2-[2-[ethoxy]ethoxy]acetic acid
  VARIANT (9)..(9): des-Xaa, Cys, or selenocysteine
  VARIANT (10)..(10): des-Xaa, Arg, citrulline, or omega-nitro-Arg
  VARIANT (11)..(11): des-Xaa, Tyr, or mono-iodo-Tyr
  VARIANT (12)..(12): des-Xaa, Arg, or Gln
  VARIANT (13)..(13): des-Xaa, Cys, or selenocysteine
  VARIANT (14)..(14): des-Xaa, Arg, Tyr, Phe, Trp, Tyr-Tyr, Tyr-Arg, Arg-Arg-Arg, Arg-Arg, Arg-Tyr, Arg-Arg-Tyr, or Tyr-Arg-Arg
XXXXDXPRXXXXXX

SEQ ID NO: 180 - protein, 14 aa, Artificial sequence
  RgIA analog
  VARIANT (1)..(1): des-Xaa or Gly
  VARIANT (2)..(2): des-Xaa, Cys, or selenocysteine
  VARIANT (3)..(3): des-Xaa, Cys, or selenocysteine
  VARIANT (4)..(4): des-Xaa, Ser, or Thr
  MISC_FEATURE (7)..(7): 2-[2-[ethoxy]ethoxy]acetic acid
  VARIANT (9)..(9): des-Xaa, Cys, or selenocysteine
  VARIANT (10)..(10): des-Xaa, Arg, citrulline, or omega-nitro-Arg
  VARIANT (11)..(11): des-Xaa, Tyr, or mono-iodo-Tyr
  VARIANT (12)..(12): des-Xaa, Arg, or Gln
  VARIANT (13)..(13): des-Xaa, Cys, or selenocysteine
  VARIANT (14)..(14): des-Xaa, Arg, Tyr, Phe, Trp, Tyr-Tyr, Tyr-Arg, Arg-Arg-Arg, Arg-Arg, Arg-Tyr, Arg-Arg-Tyr, or Tyr-Arg-Arg
XXXXDPXRXXXXXX

SEQ ID NO: 181 - protein, 14 aa, Artificial sequence
  RgIA analog
  VARIANT (1)..(1): des-Xaa or Gly
  VARIANT (2)..(2): des-Xaa, Cys, or selenocysteine
  VARIANT (3)..(3): des-Xaa, Cys, or selenocysteine
  VARIANT (4)..(4): des-Xaa, Ser, or Thr
  MISC_FEATURE (8)..(8): 2-[2-[ethoxy]ethoxy]acetic acid
  VARIANT (9)..(9): des-Xaa, Cys, or selenocysteine
  VARIANT (10)..(10): des-Xaa, Arg, citrulline, or omega-nitro-Arg
  VARIANT (11)..(11): des-Xaa, Tyr, or mono-iodo-Tyr
  VARIANT (12)..(12): des-Xaa, Arg, or Gln
  VARIANT (13)..(13): des-Xaa, Cys, or selenocysteine
  VARIANT (14)..(14): des-Xaa, Arg, Tyr, Phe, Trp, Tyr-Tyr, Tyr-Arg, Arg-Arg-Arg, Arg-Arg, Arg-Tyr, Arg-Arg-Tyr, or Tyr-Arg-Arg
XXXXDPRXXXXXXX

SEQ ID NO: 182 - protein, 14 aa, Artificial sequence
  RgIA analog
  VARIANT (1)..(1): des-Xaa or Gly
  VARIANT (2)..(2): des-Xaa, Cys, or selenocysteine
  VARIANT (3)..(3): des-Xaa, Cys, or selenocysteine
  VARIANT (4)..(4): des-Xaa, Ser, or Thr
  MISC_FEATURE (5)..(5): 2-[2-[2-[ethoxy]ethoxy]ethoxy]acetic acid
  VARIANT (9)..(9): des-Xaa, Cys, or selenocysteine
  VARIANT (10)..(10): des-Xaa, Arg, citrulline, or omega-nitro-Arg
  VARIANT (11)..(11): des-Xaa, Tyr, or mono-iodo-Tyr
  VARIANT (12)..(12): des-Xaa, Arg, or Gln
  VARIANT (13)..(13): des-Xaa, Cys, or selenocysteine
  VARIANT (14)..(14): des-Xaa, Arg, Tyr, Phe, Trp, Tyr-Tyr, Tyr-Arg, Arg-Arg-Arg, Arg-Arg, Arg-Tyr, Arg-Arg-Tyr, or Tyr-Arg-Arg
XXXXXDPRXXXXXX

SEQ ID NO: 183 - protein, 14 aa, Artificial sequence
  RgIA analog
  VARIANT (1)..(1): des-Xaa or Gly
  VARIANT (2)..(2): des-Xaa, Cys, or selenocysteine
  VARIANT (3)..(3): des-Xaa, Cys, or selenocysteine
  VARIANT (4)..(4): des-Xaa, Ser, or Thr
  MISC_FEATURE (6)..(6): 2-[2-[2-[ethoxy]ethoxy]ethoxy]acetic acid
  VARIANT (9)..(9): des-Xaa, Cys, or selenocysteine
  VARIANT (10)..(10): des-Xaa, Arg, citrulline, or omega-nitro-Arg
  VARIANT (11)..(11): des-Xaa, Tyr, or mono-iodo-Tyr
  VARIANT (12)..(12): des-Xaa, Arg, or Gln
  VARIANT (13)..(13): des-Xaa, Cys, or selenocysteine
  VARIANT (14)..(14): des-Xaa, Arg, Tyr, Phe, Trp, Tyr-Tyr, Tyr-Arg, Arg-Arg-Arg, Arg-Arg, Arg-Tyr, Arg-Arg-Tyr, or Tyr-Arg-Arg
XXXXDXPRXXXXXX

SEQ ID NO: 184 - protein, 14 aa, Artificial sequence
  RgIA analog
  VARIANT (1)..(1): des-Xaa or Gly
  VARIANT (2)..(2): des-Xaa, Cys, or selenocysteine
  VARIANT (3)..(3): des-Xaa, Cys, or selenocysteine
  VARIANT (4)..(4): des-Xaa, Ser, or Thr
  MISC_FEATURE (7)..(7): 2-[2-[2-[ethoxy]ethoxy]ethoxy]acetic acid
  VARIANT (9)..(9): des-Xaa, Cys, or selenocysteine
  VARIANT (10)..(10): des-Xaa, Arg, citrulline, or omega-nitro-Arg
  VARIANT (11)..(11): des-Xaa, Tyr, or mono-iodo-Tyr
  VARIANT (12)..(12): des-Xaa, Arg, or Gln
  VARIANT (13)..(13): des-Xaa, Cys, or selenocysteine
  VARIANT (14)..(14): des-Xaa, Arg, Tyr, Phe, Trp, Tyr-Tyr, Tyr-Arg, Arg-Arg-Arg, Arg-Arg, Arg-Tyr, Arg-Arg-Tyr, or Tyr-Arg-Arg
XXXXDPXRXXXXXX

SEQ ID NO: 185 - protein, 14 aa, Artificial sequence
  RgIA analog
  VARIANT (1)..(1): des-Xaa or Gly
  VARIANT (2)..(2): des-Xaa, Cys, or selenocysteine
  VARIANT (3)..(3): des-Xaa, Cys, or selenocysteine
  VARIANT (4)..(4): des-Xaa, Ser, or Thr
  MISC_FEATURE (8)..(8): 2-[2-[2-[ethoxy]ethoxy]ethoxy]acetic acid
  VARIANT (9)..(9): des-Xaa, Cys, or selenocysteine
  VARIANT (10)..(10): des-Xaa, Arg, citrulline, or omega-nitro-Arg
  VARIANT (11)..(11): des-Xaa, Tyr, or mono-iodo-Tyr
  VARIANT (12)..(12): des-Xaa, Arg, or Gln
  VARIANT (13)..(13): des-Xaa, Cys, or selenocysteine
  VARIANT (14)..(14): des-Xaa, Arg, Tyr, Phe, Trp, Tyr-Tyr, Tyr-Arg, Arg-Arg-Arg, Arg-Arg, Arg-Tyr, Arg-Arg-Tyr, or Tyr-Arg-Arg
XXXXDPRXXXXXXX

SEQ ID NO: 186 - protein, 13 aa, Artificial sequence
  RgIA analog
  MOD_RES (1)..(1): Acylation
GCCSDPRCRYRCR

SEQ ID NO: 187 - protein, 13 aa, Artificial sequence
  RgIA analog
  MOD_RES (1)..(1): Acylation
  VARIANT (10)..(10): des-Xaa, Ser, or Thr
GCCSDPRCRXRCR

SEQ ID NO: 188 - protein, 13 aa, Artificial sequence
  RgIA analog
  MOD_RES (1)..(1): Acylation
  VARIANT (9)..(9): des-Xaa, Tyr, or mono-iodo-Tyr
  VARIANT (10)..(10): des-Xaa, Ser, or Thr
GCCTDPRCXXQCR

SEQ ID NO: 189 - protein, 15 aa, Artificial sequence
  RgIA analog
  MOD_RES (1)..(1): Acylation
  VARIANT (9)..(9): des-Xaa, Tyr, or mono-iodo-Tyr
  VARIANT (10)..(10): des-Xaa, Ser, or Thr
GCCTDPRCXXQCRRR

SEQ ID NO: 190 - protein, 13 aa, Artificial sequence
  RgIA analog
  MOD_RES (1)..(1): Acylation
  VARIANT (9)..(9): des-Xaa, Tyr, or mono-iodo-Tyr
  VARIANT (10)..(10): des-Xaa, Ser, or Thr
GCCTDPRCXXQCY

SEQ ID NO: 191 - protein, 13 aa, Artificial sequence
  RgIA analog
  MOD_RES (1)..(1): Acylation
  VARIANT (2)..(2): des-Xaa, Arg, or Gln
  VARIANT (8)..(8): des-Xaa, Arg, or Gln
  VARIANT (9)..(9): des-Xaa, Tyr, or mono-iodo-Tyr
  VARIANT (10)..(10): des-Xaa, Ser, or Thr
GXCTDPRXXXQCR

SEQ ID NO: 192 - protein, 13 aa, Artificial sequence
  RgIA analog
  MOD_RES (1)..(1): Acylation
  VARIANT (10)..(10): des-Xaa, Ser, or Thr
GCCTDPRCRXQCF

SEQ ID NO: 193 - protein, 13 aa, Artificial sequence
  RgIA analog
  MOD_RES (1)..(1): Acylation
  VARIANT (10)..(10): des-Xaa, Ser, or Thr
GCCTDPRCRXQCY

SEQ ID NO: 194 - protein, 13 aa, Artificial sequence
  RgIA analog
  MOD_RES (1)..(1): Acylation
  VARIANT (10)..(10): des-Xaa, Ser, or Thr
GCCTDPRCRXQCW

SEQ ID NO: 195 - protein, 13 aa, Artificial sequence
  RgIA analog
  MOD_RES (1)..(1): Acylation
  MOD_RES (13)..(13): AMIDATION
GCCSDPRCRYRCR

SEQ ID NO: 196 - protein, 13 aa, Artificial sequence
  RgIA analog
  MOD_RES (1)..(1): Acylation
  VARIANT (10)..(10): des-Xaa, Ser, or Thr
  MOD_RES (13)..(13): AMIDATION
GCCSDPRCRXRCR

SEQ ID NO: 197 - protein, 13 aa, Artificial sequence
  RgIA analog
  MOD_RES (1)..(1): Acylation
  VARIANT (9)..(9): des-Xaa, Tyr, or mono-iodo-Tyr
  VARIANT (10)..(10): des-Xaa, Ser, or Thr
  MOD_RES (13)..(13): AMIDATION
GCCTDPRCXXQCR

SEQ ID NO: 198 - protein, 15 aa, Artificial sequence
  RgIA analog
  MOD_RES (1)..(1): Acylation
  VARIANT (9)..(9): des-Xaa, Tyr, or mono-iodo-Tyr
  VARIANT (10)..(10): des-Xaa, Ser, or Thr
  MOD_RES (15)..(15): AMIDATION
GCCTDPRCXXQCRRR

SEQ ID NO: 199 - protein, 13 aa, Artificial sequence
  RgIA analog
  MOD_RES (1)..(1): Acylation
  VARIANT (9)..(9): des-Xaa, Tyr, or mono-iodo-Tyr
  VARIANT (10)..(10): des-Xaa, Ser, or Thr
  MOD_RES (13)..(13): AMIDATION
GCCTDPRCXXQCY

SEQ ID NO: 200 - protein, 13 aa, Artificial sequence
  RgIA analog
  MOD_RES (1)..(1): Acylation
  VARIANT (2)..(2): des-Xaa, Arg, or Gln
  VARIANT (8)..(8): des-Xaa, Arg, or Gln
  VARIANT (9)..(9): des-Xaa, Tyr, or mono-iodo-Tyr
  VARIANT (10)..(10): des-Xaa, Ser, or Thr
  MOD_RES (13)..(13): AMIDATION
GXCTDPRXXXQCR

SEQ ID NO: 201 - protein, 13 aa, Artificial sequence
  RgIA analog
  MOD_RES (1)..(1): Acylation
  VARIANT (10)..(10): des-Xaa, Ser, or Thr
  MOD_RES (13)..(13): AMIDATION
GCCTDPRCRXQCF

SEQ ID NO: 202 - protein, 13 aa, Artificial sequence
  RgIA analog
  MOD_RES (1)..(1): Acylation
  VARIANT (10)..(10): des-Xaa, Ser, or Thr
  MOD_RES (13)..(13): AMIDATION
GCCTDPRCRXQCY

SEQ ID NO: 203 - protein, 13 aa, Artificial sequence
  RgIA analog
  MOD_RES (1)..(1): Acylation
  VARIANT (10)..(10): des-Xaa, Ser, or Thr
  MOD_RES (13)..(13): AMIDATION
GCCTDPRCRXQCW

SEQ ID NO: 204 - protein, 13 aa, Artificial sequence
  RgIA analog
  MOD_RES (1)..(1): Acylation
  MOD_RES (13)..(13): D-isomer
GCCSDPRCRYRCR

SEQ ID NO: 205 - protein, 13 aa, Artificial sequence
  RgIA analog
  MOD_RES (1)..(1): Acylation
  VARIANT (10)..(10): des-Xaa, Ser, or Thr
  MOD_RES (13)..(13): D-isomer
GCCSDPRCRXRCR

SEQ ID NO: 206 - protein, 13 aa, Artificial sequence
  RgIA analog
  MOD_RES (1)..(1): Acylation
  VARIANT (9)..(9): des-Xaa, Tyr, or mono-iodo-Tyr
  VARIANT (10)..(10): des-Xaa, Ser, or Thr
  MOD_RES (13)..(13): D-isomer
GCCTDPRCXXQCR

SEQ ID NO: 207 - protein, 15 aa, Artificial sequence
  RgIA analog
  MOD_RES (1)..(1): Acylation
  VARIANT (9)..(9): des-Xaa, Tyr, or mono-iodo-Tyr
  VARIANT (10)..(10): des-Xaa, Ser, or Thr
  MOD_RES (15)..(15): D-isomer
GCCTDPRCXXQCRRR

SEQ ID NO: 208 - protein, 13 aa, Artificial sequence
  RgIA analog
  MOD_RES (1)..(1): Acylation
  VARIANT (9)..(9): des-Xaa, Tyr, or mono-iodo-Tyr
  VARIANT (10)..(10): des-Xaa, Ser, or Thr
  MOD_RES (13)..(13): D-isomer
GCCTDPRCXXQCY

SEQ ID NO: 209 - protein, 13 aa, Artificial sequence
  RgIA analog
  MOD_RES (1)..(1): Acylation
  VARIANT (2)..(2): des-Xaa, Arg, or Gln
  VARIANT (8)..(8): des-Xaa, Arg, or Gln
  VARIANT (9)..(9): des-Xaa, Tyr, or mono-iodo-Tyr
  VARIANT (10)..(10): des-Xaa, Ser, or Thr
  MOD_RES (13)..(13): D-isomer
GXCTDPRXXXQCR

SEQ ID NO: 210 - protein, 13 aa, Artificial sequence
  RgIA analog
  MOD_RES (1)..(1): Acylation
  VARIANT (10)..(10): des-Xaa, Ser, or Thr
  MOD_RES (13)..(13): D-isomer
GCCTDPRCRXQCF

SEQ ID NO: 211 - protein, 13 aa, Artificial sequence
  RgIA analog
  MOD_RES (1)..(1): Acylation
  VARIANT (10)..(10): des-Xaa, Ser, or Thr
  MOD_RES (13)..(13): D-isomer
GCCTDPRCRXQCY

SEQ ID NO: 212 - protein, 13 aa, Artificial sequence
  RgIA analog
  MOD_RES (1)..(1): Acylation
  VARIANT (10)..(10): des-Xaa, Ser, or Thr
  MOD_RES (13)..(13): D-isomer
GCCTDPRCRXQCW

SEQ ID NO: 213 - protein, 13 aa, Artificial sequence
  RgIA analog
  MOD_RES (1)..(1): Acylation
  MOD_RES (13)..(13): D-isomer
  MOD_RES (13)..(13): AMIDATION
GCCSDPRCRYRCR

SEQ ID NO: 214 - protein, 13 aa, Artificial sequence
  RgIA analog
  MOD_RES (1)..(1): Acylation
  VARIANT (10)..(10): des-Xaa, Ser, or Thr
  MOD_RES (13)..(13): D-isomer
  MOD_RES (13)..(13): AMIDATION
GCCSDPRCRXRCR

SEQ ID NO: 215 - protein, 13 aa, Artificial sequence
  RgIA analog
  MOD_RES (1)..(1): Acylation
  VARIANT (9)..(9): des-Xaa, Tyr, or mono-iodo-Tyr
  VARIANT (10)..(10): des-Xaa, Ser, or Thr
  MOD_RES (13)..(13): D-isomer
  MOD_RES (13)..(13): AMIDATION
GCCTDPRCXXQCR

SEQ ID NO: 216 - protein, 15 aa, Artificial sequence
  RgIA analog
  MOD_RES (1)..(1): Acylation
  VARIANT (9)..(9): des-Xaa, Tyr, or mono-iodo-Tyr
  VARIANT (10)..(10): des-Xaa, Ser, or Thr
  MOD_RES (15)..(15): D-isomer
  MOD_RES (15)..(15): AMIDATION
GCCTDPRCXXQCRRR

SEQ ID NO: 217 - protein, 13 aa, Artificial sequence
  RgIA analog
  MOD_RES (1)..(1): Acylation
  VARIANT (9)..(9): des-Xaa, Tyr, or mono-iodo-Tyr
  VARIANT (10)..(10): des-Xaa, Ser, or Thr
  MOD_RES (13)..(13): D-isomer
  MOD_RES (13)..(13): AMIDATION
GCCTDPRCXXQCR

SEQ ID NO: 218 - protein, 13 aa, Artificial sequence
  RgIA analog
  MOD_RES (1)..(1): Acylation
  VARIANT (2)..(2): des-Xaa, Arg, or Gln
  VARIANT (8)..(8): des-Xaa, Arg, or Gln
  VARIANT (9)..(9): des-Xaa, Tyr, or mono-iodo-Tyr
  VARIANT (10)..(10): des-Xaa, Ser, or Thr
  MOD_RES (13)..(13): D-isomer
  MOD_RES (13)..(13): AMIDATION
GXCTDPRXXXQCR

SEQ ID NO: 219 - protein, 13 aa, Artificial sequence
  RgIA analog
  MOD_RES (1)..(1): Acylation
  VARIANT (10)..(10): des-Xaa, Ser, or Thr
  MOD_RES (13)..(13): D-isomer
  MOD_RES (13)..(13): AMIDATION
GCCTDPRCRXQCF

SEQ ID NO: 220 - protein, 13 aa, Artificial sequence
  RgIA analog
  MOD_RES (1)..(1): Acylation
  VARIANT (10)..(10): des-Xaa, Ser, or Thr
  MOD_RES (13)..(13): D-isomer
  MOD_RES (13)..(13): AMIDATION
GCCTDPRCRXQCY

SEQ ID NO: 221 - protein, 13 aa, Artificial sequence
  RgIA analog
  MOD_RES (1)..(1): Acylation
  VARIANT (10)..(10): des-Xaa, Ser, or Thr
  MOD_RES (13)..(13): D-isomer
  MOD_RES (13)..(13): AMIDATION
GCCTDPRCRXQCW

SEQ ID NO: 222 - protein, 15 aa, Artificial sequence
  RgIA analog
  MOD_RES (9)..(9): 7-carboxy-Glu
  MOD_RES (10)..(10): 3-iodo-Tyrosine
GCCTDPRCXXQCYRR

SEQ ID NO: 223 - protein, 15 aa, Artificial sequence
  RgIA analog
  MOD_RES (9)..(9): 7-carboxy-Glu
  MOD_RES (10)..(10): 3-iodo-Tyrosine
GCCTDPRCXXQCRRY

SEQ ID NO: 224 - protein, 13 aa, Artificial sequence
  RgIA analog
  MOD_RES (9)..(9): 7-carboxy-Glu
  MOD_RES (10)..(10): 3-iodo-Tyrosine
GCCTDPRCXXQCF

SEQ ID NO: 225 - protein, 13 aa, Artificial sequence
  RgIA analog
  MOD_RES (9)..(9): 7-carboxy-Glu
  MOD_RES (10)..(10): 3-iodo-Tyrosine
GCCTDPRCXXQCW

SEQ ID NO: 226 - protein, 14 aa, Artificial sequence
  RgIA analog
  MOD_RES (9)..(9): 7-carboxy-Glu
  MOD_RES (10)..(10): 3-iodo-Tyrosine
GCCTDPRCXXQCYY

SEQ ID NO: 227 - protein, 14 aa, Artificial sequence
  RgIA analog
  MOD_RES (9)..(9): 7-carboxy-Glu
  MOD_RES (10)..(10): 3-iodo-Tyrosine
GCCTDPRCXXQCYR

SEQ ID NO: 228 - protein, 15 aa, Artificial sequence
  RgIA analog
  MOD_RES (10)..(10): 3-iodo-Tyrosine
GCCTDPRCRXQCRRR

SEQ ID NO: 229 - protein, 15 aa, Artificial sequence
  RgIA analog
  MOD_RES (10)..(10): 3-iodo-Tyrosine
GCCTDPRCRXQCYRR

SEQ ID NO: 230 - protein, 15 aa, Artificial sequence
  RgIA analog
  MOD_RES (10)..(10): 3-iodo-Tyrosine
GCCTDPRCRXQCRRY

SEQ ID NO: 231 - protein, 14 aa, Artificial sequence
  RgIA analog
  MOD_RES (10)..(10): 3-iodo-Tyrosine
GCCTDPRCRXQCYY

SEQ ID NO: 232 - protein, 14 aa, Artificial sequence
  RgIA analog
  MOD_RES (10)..(10): 3-iodo-Tyrosine
GCCTDPRCRXQCYR

SEQ ID NO: 233 - protein, 16 aa, Artificial sequence
  RgIA analog
GCCSDPRCNYDHPEIC

SEQ ID NO: 234 - protein, 16 aa, Artificial sequence
  RgIA analog
  MOD_RES (16)..(16): AMIDATION
GCCSDPRCNYDHPEIC

SEQ ID NO: 235 - protein, 16 aa, Artificial sequence
  RgIA analog
GCCSHPACSVNHPELC

SEQ ID NO: 236 - protein, 16 aa, Artificial sequence
  RgIA analog
  MOD_RES (16)..(16): AMIDATION
GCCSHPACSVNHPELC

SEQ ID NO: 237 - protein, 13 aa, Artificial sequence
  RgIA analog
GCCTDPRCRYRCR

SEQ ID NO: 238 - protein, 14 aa, Artificial sequence
  RgIA analog
  MOD_RES (6)..(6): hydroxy-Pro
GCCSDXQRCRYRCR

SEQ ID NO: 239 - protein, 13 aa, Artificial sequence
  RgIA analog
  MOD_RES (6)..(6): hydroxy-Pro
GCCTDXRCRYRCR

SEQ ID NO: 240 - protein, 13 aa, Artificial sequence
  RgIA analog
  MOD_RES (10)..(10): mono-halo Tyr
GCCSDPRCRXRCR

SEQ ID NO: 241 - protein, 13 aa, Artificial sequence
  RgIA analog
  MOD_RES (10)..(10): mono-halo Tyr
GCCTDPRCRXRCR

SEQ ID NO: 242 - protein, 14 aa, Artificial sequence
  RgIA analog
  MOD_RES (1)..(1): mono-halo Tyr
  MOD_RES (7)..(7): hydroxy-Pro
  MOD_RES (11)..(11): mono-halo Tyr
XGCCSDXRCRXRCR

SEQ ID NO: 243 - protein, 14 aa, Artificial sequence
  RgIA analog
  MOD_RES (1)..(1): mono-halo Tyr
  MOD_RES (7)..(7): hydroxy-Pro
  MOD_RES (11)..(11): mono-halo Tyr
XGCCTDXRCRXRCR

SEQ ID NO: 244 - protein, 13 aa, Artificial sequence
  RgIA analog
  VARIANT (9)..(9): homo-Arg or ornithine
GCCSDPRCXYRCR

SEQ ID NO: 245 - protein, 13 aa, Artificial sequence
  RgIA analog
  MOD_RES (9)..(9): 7-carboxy-Glu
  MOD_RES (10)..(10): 3-iodo-Tyrosine
GCCSDPRCXXRCR

SEQ ID NO: 246 - protein, 13 aa, Artificial sequence
  RgIA analog
  MOD_RES (2)..(2): Selenocysteine
  MOD_RES (8)..(8): Selenocysteine
  MOD_RES (9)..(9): 7-carboxy-Glu
  MOD_RES (10)..(10): 3-iodo-Tyrosine
GXCTDPRXXXQCK

SEQ ID NO: 247 - protein, 13 aa, Artificial sequence
  RgIA analog
  MOD_RES (2)..(2): Selenocysteine
  MOD_RES (8)..(8): Selenocysteine
GXCSDPRXRYRCR

SEQ ID NO: 248 - protein, 13 aa, Artificial sequence
  RgIA analog
  MOD_RES (9)..(9)
  MOD_RES (10)..(10): 3-iodo-Tyrosine
GCCTDPRCXXRCR

SEQ ID NO: 249 - protein, 13 aa, Artificial sequence
  RgIA analog
  MOD_RES (9)..(9): 7-carboxy-Glu
GCCSDPRCXYRCR

SEQ ID NO: 250 - protein, 13 aa, Artificial sequence
  RgIA analog
GCCSDPRCRYQCR

SEQ ID NO: 251 - protein, 13 aa, Artificial sequence
  RgIA analog
GCCSDPRCFWRCR

SEQ ID NO: 252 - protein, 13 aa, Artificial sequence
  RgIA analog
  MOD_RES (2)..(2): homocysteine
GXCSDPRCRYRCR

SEQ ID NO: 253 - protein, 13 aa, Artificial sequence
  RgIA analog
GCCADPRCRYRCR

SEQ ID NO: 254 - protein, 13 aa, Artificial sequence
  RgIA analog
GCCYDPRCRYRCR

SEQ ID NO: 255 - protein, 13 aa, Artificial sequence
  RgIA analog
  MOD_RES (8)..(8): homocysteine
GCCSDPRXRYRCR

SEQ ID NO: 256 - protein, 13 aa, Artificial sequence
  RgIA analog
GCCSDPRCGYRCR

SEQ ID NO: 257 - protein, 13 aa, Artificial sequence
  RgIA analog
GCCSDPRCAYRCR

SEQ ID NO: 258 - protein, 13 aa, Artificial sequence
  RgIA analog
GCCSDPRCVYRCR

SEQ ID NO: 259 - protein, 13 aa, Artificial sequence
  RgIA analog
GCCSDPRCLYRCR

SEQ ID NO: 260 - protein, 13 aa, Artificial sequence
  RgIA analog
GCCSDPRCIYRCR

SEQ ID NO: 261 - protein, 13 aa, Artificial sequence
  RgIA analog
GCCSDPRCMYRCR

SEQ ID NO: 262 - protein, 13 aa, Artificial sequence
  RgIA analog
GCCSDPRCFYRCR

SEQ ID NO: 263 - protein, 13 aa, Artificial sequence
  RgIA analog
GCCSDPRCWYRCR

SEQ ID NO: 264 - protein, 13 aa, Artificial sequence
  RgIA analog
GCCSDPRCPYRCR

SEQ ID NO: 265 - protein, 13 aa, Artificial sequence
  RgIA analog
GCCSDPRCSYRCR

SEQ ID NO: 266 - protein, 13 aa, Artificial sequence
  RgIA analog
GCCSDPRCTYRCR

SEQ ID NO: 267 - protein, 13 aa, Artificial sequence
  RgIA analog
GCCSDPRCCYRCR

SEQ ID NO: 268 - protein, 13 aa, Artificial sequence
  RgIA analog
GCCSDPRCYYRCR

SEQ ID NO: 269 - protein, 13 aa, Artificial sequence
  RgIA analog
GCCSDPRCNYRCR

SEQ ID NO: 270 - protein, 13 aa, Artificial sequence
  RgIA analog
GCCSDPRCQYRCR

SEQ ID NO: 271 - protein, 13 aa, Artificial sequence
  RgIA analog
GCCSDPRCDYRCR

SEQ ID NO: 272 - protein, 13 aa, Artificial sequence
  RgIA analog
GCCSDPRCEYRCR

SEQ ID NO: 273 - protein, 13 aa, Artificial sequence
  RgIA analog
GCCSDPRCKYRCR

SEQ ID NO: 274 - protein, 13 aa, Artificial sequence
  RgIA analog
GCCSDPRCHYRCR

SEQ ID NO: 275 - protein, 13 aa, Artificial sequence
  RgIA analog
GCCSDPRCRFRCR

SEQ ID NO: 276 - protein, 13 aa, Artificial sequence
  RgIA analog
GCCSDPRCRYHCR

SEQ ID NO: 277 - protein, 13 aa, Artificial sequence
  RgIA analog
  MOD_RES (9)..(9): omega-nitro-Arg
  MOD_RES (10)..(10): 3-iodo-Tyrosine
GCCSDPRCXXRCR

SEQ ID NO: 278 - protein, 12 aa, Artificial sequence
  RgIA analog
GCCSDPRCRYRC

SEQ ID NO: 279 - protein, 13 aa, Artificial sequence
  RgIA analog
GCCSEPRCRYRCR

SEQ ID NO: 280 - protein, 13 aa, Artificial sequence
  RgIA analog
GCCSDVRCRYRCR

SEQ ID NO: 281 - protein, 13 aa, Artificial sequence
  RgIA analog
GCCSDPRCAYRCR

SEQ ID NO: 282 - protein, 13 aa, Artificial sequence
  RgIA analog
GCCSHPACRYRCR

SEQ ID NO: 283 - protein, 13 aa, Artificial sequence
  RgIA analog
  MOD_RES (9)..(9): D-Arg
GCCSDPRCXYRCR

SEQ ID NO: 284 - protein, 12 aa, Artificial sequence
  RgIA analog
ACCSDRRCRWRC

SEQ ID NO: 285 - protein, 35 aa, Artificial sequence
  RgIA analog
FDGRNAPADDKASDLIAQIVRRACCSDRRCRWRCG

SEQ ID NO: 286 - protein, 13 aa, Artificial sequence
  RgIA analog
  MOD_RES (1)..(1): mono-halo Tyr
  MOD_RES (6)..(6): hydroxy-Pro
  MOD_RES (10)..(10): mono-halo Tyr
XGCCSXRCRXRCR

SEQ ID NO: 287 - protein, 32 aa, Artificial sequence
  RgIA analog
SNKRKNAAMLDMIAQHAIRGCCSDPRCRYRCR

SEQ ID NO: 288 - protein, 16 aa, Artificial sequence
  RgIA analog
DECCSNPACRVNNPHV

SEQ ID NO: 289 - protein, 39 aa, Artificial sequence
  RgIA analog
SDGRNVAAKAFHRIGRTIRDECCSNPACRVNNPHVCRRR

SEQ ID NO: 290 - protein, 20 aa, Artificial sequence
  RgIA analog
DECCSNPACRLNNPHACRRR

SEQ ID NO: 291 - protein, 20 aa, Artificial sequence
  RgIA analog
  MOD_RES (2)..(2): gamma-carboxy-Glu (Gla)
DXCCSNPACRLNNPHACRRR

SEQ ID NO: 292 - protein, 20 aa, Artificial sequence
  RgIA analog
  MOD_RES (7)..(7): hydroxy-Pro
DECCSNXACRLNNPHACRRR

SEQ ID NO: 293 - protein, 21 aa, Artificial sequence
  RgIA analog
  MOD_RES (1)..(1): gamma-carboxy-Glu (Gla)
  MOD_RES (3)..(3): gamma-carboxy-Glu (Gla)
  MOD_RES (8)..(8): hydroxy-Pro
XDXCCSNXACRLNNPHACRRR

SEQ ID NO: 294 - protein, 20 aa, Artificial sequence
  RgIA analog
  MOD_RES (14)..(14): hydroxy-Pro
DECCSNPACRLNNXHACRRR

SEQ ID NO: 295 - protein, 20 aa, Artificial sequence
  RgIA analog
  MOD_RES (1)..(1): gamma-carboxy-Glu (Gla)
  MOD_RES (3)..(3): gamma-carboxy-Glu (Gla)
  MOD_RES (14)..(14): hydroxy-Pro
XDXCCSNPACRLNXHACRRR

SEQ ID NO: 296 - protein, 20 aa, Artificial sequence
  RgIA analog
  MOD_RES (7)..(7): hydroxy-Pro
  MOD_RES (14)..(14): hydroxy-Pro
DECCSNXACRLNNXHACRRR

SEQ ID NO: 297 - protein, 21 aa, Artificial sequence
  RgIA analog
  MOD_RES (1)..(1): gamma-carboxy-Glu (Gla)
  MOD_RES (3)..(3): gamma-carboxy-Glu (Gla)
  MOD_RES (8)..(8): hydroxy-Pro
  MOD_RES (15)..(15): hydroxy-Pro
XDXCCSNXACRLNNXHACRRR

SEQ ID NO: 298 - protein, 20 aa, Artificial sequence
  RgIA analog
DECCSNPACRLNNPHVCRRR

SEQ ID NO: 299 - protein, 20 aa, Artificial sequence
  RgIA analog
  MOD_RES (2)..(2): gamma-carboxy-Glu (Gla)
DXCCSNPACRLNNPHVCRRR

SEQ ID NO: 300 - protein, 20 aa, Artificial sequence
  RgIA analog
  MOD_RES (7)..(7): gamma-carboxy-Glu (Gla)
DECCSNXACRLNNPHVCRRR

SEQ ID NO: 301 - protein, 20 aa, Artificial sequence
  RgIA analog
  MOD_RES (1)..(1): gamma-carboxy-Glu (Gla)
  MOD_RES (3)..(3): gamma-carboxy-Glu (Gla)
  MOD_RES (8)..(8): hydroxy-Pro
XDXCCSNXACRLNPHVCRRR

SEQ ID NO: 302 - protein, 20 aa, Artificial sequence
  RgIA analog
  MOD_RES (14)..(14): hydroxy-Pro
DECCSNPACRLNNXHVCRRR

SEQ ID NO: 303 - protein, 21 aa, Artificial sequence
  RgIA analog
  MOD_RES (1)..(1): gamma-carboxy-Glu (Gla)
  MOD_RES (3)..(3): gamma-carboxy-Glu (Gla)
  MOD_RES (8)..(8): hydroxy-Pro
XDXCCSNXACRLNNPHVCRRR

SEQ ID NO: 304 - protein, 20 aa, Artificial sequence
  RgIA analog
  MOD_RES (7)..(7): hydroxy-Pro
  MOD_RES (14)..(14): hydroxy-Pro
DECCSNXACRLNNXHVCRRR

SEQ ID NO: 305 - protein, 21 aa, Artificial sequence
  RgIA analog
  MOD_RES (1)..(1): gamma-carboxy-Glu (Gla)
  MOD_RES (3)..(3): gamma-carboxy-Glu (Gla)
  MOD_RES (8)..(8): hydroxy-Pro
  MOD_RES (15)..(15): hydroxy-Pro
XDXCCSNXACRLNNXHVCRRR

SEQ ID NO: 306 - protein, 16 aa, Artificial sequence
  RgIA analog
GCCSHPACNVDHPEIC

SEQ ID NO: 307 - protein, 64 aa, Artificial sequence
  RgIA analog
MFTVFLLVVLATTVVSFTSDRAFRGRNSAANDKRSDLAALSVRRGCCSHPACSVNHPELCGRRR

SEQ ID NO: 308 - protein, 21 aa, Artificial sequence
  RgIA analog
ECCTNPVCHAEHQHELCARRR

SEQ ID NO: 309 - protein, 20 aa, Artificial sequence
  RgIA analog
  MOD_RES (11)..(11): 7-carboxy-Glu
ECCTNPVCHAXHQELCARRR

SEQ ID NO: 310 - protein, 20 aa, Artificial sequence
  RgIA analog
  MOD_RES (11)..(11): 7-carboxy-Glu
  MOD_RES (14)..(14): 7-carboxy-Glu
ECCTNPVCHAXHQXLCARRR

SEQ ID NO: 311 - protein, 20 aa, Artificial sequence
  RgIA analog
  MOD_RES (11)..(11): 3-iodo-Tyrosine
  MOD_RES (14)..(14): 7-carboxy-Glu
ECCTNPVCHAXHQXLCARRR

SEQ ID NO: 312 - protein, 21 aa, Artificial sequence
  RgIA analog
  MOD_RES (1)..(1): 7-carboxy-Glu
XCCTNPVCHAEHQHELCARRR

SEQ ID NO: 313 - protein, 20 aa, Artificial sequence
  RgIA analog
  MOD_RES (1)..(1): 7-carboxy-Glu
  MOD_RES (11)..(11): 7-carboxy-Glu
XCCTNPVCHAXHQELCARRR

SEQ ID NO: 314 - protein, 20 aa, Artificial sequence
  RgIA analog
  MOD_RES (1)..(1): 7-carboxy-Glu
  MOD_RES (11)..(11): 7-carboxy-Glu
  MOD_RES (14)..(14): 7-carboxy-Glu
XCCTNPVCHAXHQXLCARRR

SEQ ID NO: 315 - protein, 20 aa, Artificial sequence
  RgIA analog
  MOD_RES (1)..(1): 7-carboxy-Glu
  MOD_RES (11)..(11): 3-iodo-Tyrosine
  MOD_RES (14)..(14): 7-carboxy-Glu
XCCTNPVCHAXHQXLCARRR

SEQ ID NO: 316 - protein, 15 aa, Artificial sequence
  RgIA analog
GCCSHPVCSAMSPIC

SEQ ID NO: 317 - protein, 15 aa, Artificial sequence
  RgIA analog
  VARIANT (13)..(13): des-Xaa, Arg, or citrulline
GCCSHPVCSAMSXIC

SEQ ID NO: 318 - protein, 15 aa, Artificial sequence
  RgIA analog
  MOD_RES (6)..(6): hydroxy-Pro
  VARIANT (13)..(13): des-Xaa, Arg, or citrulline
GCCSHXVCSAMSXIC

SEQ ID NO: 319 - protein, 15 aa, Artificial sequence
  RgIA analog
  MOD_RES (6)..(6): hydroxy-Pro
GCCSHXVCSAMSPIC